European Patent Application EP 4 273 250 A1, published November 8, 2023. Title: Recombinant microorganism expressing fucosyltransferase and Method of producing 2'-fucolsylactose using thereof. Applicant: SAMYANG CORPORATION. The sequence listing filed with the application follows.

SEQUENCE LISTING (63 sequences)

SEQ ID NO: 1 - protein, 261 aa, Artificial Sequence
  Amino acid sequence of Am2FT_2
MNMERKTGLMNKKYVSPCFLPGMRLGNIMFTLAAACAHARTVGVECRVPWAYNDASLMLRSRLGGWVLPSTPCGTNEPPSWQEPSFAYCPVPSRIRTGGLRGYFQSARYFEGQEAFIRALFAPLTAEKEPGAVGIHIRLGDYRRLRDKHRILDPGFLRRAAGHLSSGKNRLVLFSDEPDEAAEMLARVPAFGRFALEIDRGAPCESLRRMTAMEELVMSCSSFSWWGAWLGNTRKVIVPRDWFVGGVEDYRDIYLPHWVTL

SEQ ID NO: 2 - protein, 291 aa, Artificial Sequence
  Amino acid sequence of Bm2FT
MKIVQISSGLGNQLFQYALYKRLSMNNNDVFLDVETSYQLNKNQHNGYEIERIFSIQPSHATKGMIDELADVDNRLINRLRRKLFGPKNSMYTETKEFSYDCEVFTKDGIYIKGYWQNYNYFKEIEDDLKNELVFKKALDLKNSHLINQMNKEISVSIHVRRGDYYLNKEYENKFGNIADLDYYLKAINFIKKEVDDPKFYVFSDDIKWAKENLNLTDNVTYVEHNKGSDSYKDMRLMTCCKHNIIANSTFSWWGAFLNENKNKIVIAPGKWINVEGVGGINLFPEGWIVY

SEQ ID NO: 3 - protein, 299 aa, Artificial Sequence
  Amino acid sequence of Bm2FT_2
MGCIKRLFLYEYGGRCFLVIVKIKGGFGNQLFTYASAYAISQELQQNLIMDKVIYDLDYFRKFELPSLSLKYDQMLISKFVPNTKVKTLIYKVLRRLKLKGFTEVHEKKEFSFDENIYNLSGDIYLDGYWQNYRYFHKYYKDLSEMFVPRETPRKEVTDYITSLRGVNSVAMHVRRGDYKTFNGGKCLSLDYYIKAMEYFNSNDVQFYVFTDDIDFCEKNLPNSENINYVSRSEKLTDIEEFFIMKECKNFIIANSSFSWWAAYLSEQKADSLIVAPVVDMWKRDFYPDEWVALNTHLE

SEQ ID NO: 4 - protein, 287 aa, Artificial Sequence
  Amino acid sequence of Bm2FT_3
MIIVQIKGGLGNQLFSYASAYGIARENETELIIDRYIYDTSYSLRKYMLDFFPEIDEALLLKYIPKKNKISQIMYKLIRKSKLKYKYKAQLFLEEEEFKFTRISTQNENLYLNGYWQSYVYFDKYRNDIIKKFTPLVSFNQDGNQLLNEIKSYNSVAIHVRRGDYINFKGGKCLDSSYYIKAMKHLYNLKGKNLFFYIFTDDVEYCKRIFKNVANVKFIGEEAKLSDFEEFTLMTHCKNLIIGNSSFSWWAAYLASCKDKAVIAPVVDMWTEDFYLPEWIKIKADLQ

SEQ ID NO: 5 - protein, 291 aa, Artificial Sequence
  Amino acid sequence of Bs2FT
MKIVHISSGLGNQMFQYALYKKLSLIQDNVFLDTITSYQLYPNQHNGYELEKVFTIKPRHASKELTYNLSDLDNSVTSRIRRKLIGSKKSMYIEHKEFEYDPNLFYQENIYIKGYWQNYDYFKDIENELKNDFTFQRALDEKNNNLAIKINNENSISIHVRRGDYYLNRKNQEKFGDIANLEYYSKAISYIKERIDNPKFYIFSDNVEWVKQNLNSLEEAVYIDYNVGNDSYKDMQLMSLCKHNIIANSSFSWWGAFLNKNMEKIVIAPGKWINMKGVKKVNLFPKDWIIY

SEQ ID NO: 6 - protein, 289 aa, Artificial Sequence
  Amino acid sequence of Bm2FT_4
MIIVRVIGGLGNQMFQYALYKSLENEGKEVKLDLTGFGDYDLHNGYELNKIFNINENVATKDEINKLIKLPDNKVLSMIKRKFFSSTINYYSQDQFKYLSEIFQLDNVYLDGYWQSEKYFQGIKEVIRKEFKFKGEPNPKNIEMVKLMRGSNSVSIHFRRGDYISNPDAYKVHGGITTIHYYENAVKEIKSKVKEPKFFIFSDDIKWVKENFKLEDAFFIDWNTGSESYRDIELMSNCKHNIIANSTFSWWGAWLNKNKNKIVIAPNQWFNTIDTEDVIPDTWQCINTF

SEQ ID NO: 7 - protein, 308 aa, Artificial Sequence
  Amino acid sequence of Bt2FT
MNEIHVLLTGRLGNQLFQYAFARSLQKQYGGRIVCNTFDLDHRSEKSKVADQKFSYAMGDFKLDENVALEDAALPWYADFSSPLIKPVKKLFPRRYFDFMARRGYLMWQRTDYMPIPKLECEDVFAWGWWQDIRYFQDVQTELSDEVVPVTDPLPENQYIYNAASGEESVCISIRCGNYFNPTVKKLLYVCTPEYFRNAVESITKRLTHPKFIVFTDDVDWVKENIRFESAYPQYEFLYERGSDTVEEKIRMMTLCKHFIISNSTFSWWAQFLSKSENKIVIAPDRWFVDGRRIGLYMHGWTLIPAGQ

SEQ ID NO: 8 - protein, 317 aa, Artificial Sequence
  Amino acid sequence of Fp2FT
MIYVEMHGRLGNQMFQYAAARALQEKNNQPIMLSFRKVIGANTEGTAGWENSLKYFNVKPCEYYMGKKSLVTEYPVEYRLLCYAYALSYKPLMNNMNRWYEYQVKCCRFLDRFGIRWIANGYYDFHYNGLKNYLLNGSFESPKYFDSIRDKLLEEFTPREEERKENKRLYEQIRKRNSVCLSVRHFQLTGKQADMYDVCSLEYYQTAIRKMCELIENPLFVVFSDDIEWVKNTIDLSRVEVVYETPGNPVWEKLRLMYSCKNFIIPNSTFAWWAQYLSRNPDKYVLCPAKWFNNNFESPLIASQWVRIDREGNIVNE

SEQ ID NO: 9 - protein, 289 aa, Artificial Sequence
  Amino acid sequence of Gs2FT
MKIVKVIGGLGNQMFQYAFYRNLKAKFQEVKLDITAFETYKLHNGYELERVFDIKPEYATKKEIYPLTTNRNSKISKIKRRIFGGKETEYIEKDLKFDPEVFKVTGDVYFEGYWQTEKYFKEIEDLIRKDFQFKNPLTNKNLELSNKIKNENSVSIHVRRGDYYTSKKAERKHGNIATIEYYQKAVRKITEFVDNPVFYIFSDDIPWVKENLKLENEVIYVDWNKGLDSYIDMQLMSICKHNIIANSTFSWWGAWLNQNKNKIVIAPSRWINNKRLDTSDVIPKEWIKI

SEQ ID NO: 10 - protein, 314 aa, Artificial Sequence
  Amino acid sequence of Lg2FT
MLYVEMDGRCGNQLFHYAVARYIQLAIGNKEKLCLNFNKIFEKKDENNGWVDYLKDFKTVPYSYYSKSGTILKNESNFIQKIAIGLKAIQIKSLTKKSRQEQADKAEVGQRTLNKLGVYWVREGVNQIYPYKNNKILVSGICESNFIYEIQEQLQKELIPVTPVSSLNKSLLEKIDNCNSVCISVRRGDFFNNKNAKKYGVCSPEYYIRAKKYFDKKRLENTVYFCFSDDIEWCKENLKFTDKNVIFVSQEMPVYETLRLMSHCKHFILSNSTFSWWGQFLSEYKDKIVVSPARWNNDGYDTNLIDKNWILIDA

SEQ ID NO: 11 - protein, 309 aa, Artificial Sequence
  Amino acid sequence of Ll2FT
MIYVEIRGNLGNQLFIYATAKKIQKLTGQKIQLNTTTLNKYFPNYKFGLSEFIMEDPDCFIESYKKLPWFTNEYLLPIKIFKKILNKTPKINKILSDFFFKAFEKKGYFIWRGETFKKFSLGNHKNYYLSGFWQSEDYFYDIRDELLEIITPINSIRECNFELLNLIRNSESICVSIRRGDYVDNPKISAIYNVCDINYFIESVNEIKKNVVNVKVICFSDDVEWVKKNIKFDCETHYETYGNSLSEKVQLMSSCKHFVLSNSSFSWWTEFLSIRGGITIAPKNWYADEREADIYRKNWIYLEDKTEEE

SEQ ID NO: 12 - protein, 306 aa, Artificial Sequence
  Amino acid sequence of Ls2FT
MEEIHTLLTGRLGNQLFQYAFARNLQKQYGGQIYCDVYELEHRMSKVADEKFSYAMSGFKLDAGVIREDQAFPWYADFSNPVIKPIKKAMPRKYFELMARRGYLMWQRSDYMPIPVLDTQRVFASGWWQDIRYLQNVQEELSDEIVPITNPLQENRYIYDAAHDRDSVCISIRCGNYFNPTVKKLLYVCNPQYFHDSVKRISQMLAHPKFIVFTDDVSWVKEHLKFEDTYPQFEFLYERGCDTAEEKIRMMAMCNNFIISNSTFSWWAQFLSKNKEKIVIAPDKWFVDGRKIGLYMDGWTLVPAGR

SEQ ID NO: 13 - protein, 292 aa, Artificial Sequence
  Amino acid sequence of Ri2FT
MIAVKIGDGMGNQLFNYACGYAQARRDGDSLVLDISECDNSTLRDFELDKFHLKYDKKESFPNRNLGQKIYKNLRRALKYHVIKEREVYHNRDHRYDVNDIDPRVYKKKGLRNKYLYGYWQHLAYFEDYLNEITAMMTPAYEQSETVKKLQEEFKKTPTCAVHVRGGDIMGPAGAYFKHAMERMEQEKPGVRYIVFTNDMERAEEALAPVLESQKKDAVGQAENRLEFVSEMGEFSDVDEFFLMAACQNQILSNSTFSTWAAYLNQNPDKTVIMPDDLLSERMRQKNWIILK

SEQ ID NO: 14 - DNA, 786 bp, Artificial Sequence
  Nucleotide sequence encoding Am2FT_2
atgaacatggaacggaaaaccggccttatgaataaaaaatatgtttccccgtgtttcctgcccggcatgcggctgggcaacatcatgttcacgctggcggccgcctgtgcccacgcccgtaccgtaggggtggagtgccgggtgccctgggcttacaatgacgcttccctgatgctgcgctcccggctcggcggctgggtgctcccttctacgccgtgcggcaccaatgaacctccatcctggcaggaaccttcctttgcctattgtccggttccctcccgcatccggacgggcgggcttcgcggctacttccagagcgcacggtattttgaagggcaggaagcgttcatccgggcgcttttcgcgcctctcaccgcggagaaggagcccggcgccgttggcattcacatccggcttggggactacaggcgcctccgtgacaagcaccgcattctggaccctggtttcctgcggagggccgcagggcatttatcatccgggaagaaccgtctggtgctgttcagcgatgagccggacgaggcggcggagatgcttgcgcgcgtgccggcattcggacgctttgcgctggaaatcgaccgcggcgctccgtgcgaatccctccgccgcatgacggcgatggaggaactcgtcatgtcgtgttcttccttttcctggtggggcgcgtggctgggaaatacccggaaggtcatcgttccgcgcgactggtttgtcggcggtgtggaagactaccgggatatttacctgccccattgggtaacactgtaa

SEQ ID NO: 15 - DNA, 876 bp, Artificial Sequence
  Nucleotide sequence encoding Bm2FT
atgaaaattgttcagatttcttctggtctgggtaaccagctgttccagtacgccctgtacaaacgtctgtctatgaacaacaacgatgtgttcctggatgtggagacgtcttatcaactgaacaaaaatcagcacaatggttacgaaattgaacgtattttttccatccagccatcccatgctaccaagggtatgatcgatgaactggccgatgtagacaaccgtctgatcaaccgcttacgtcgtaaactgtttggtccgaaaaactctatgtataccgaaaccaaagagttcagctacgattgtgaagttttcaccaaagatggtatctatatcaagggctactggcagaactataactattttaaagagattgaagacgatctgaaaaatgaactggtctttaaaaaagctctggatctgaaaaattcgcacctgatcaatcagatgaataaagaaattagcgtaagcatccacgtacgccgcggcgattattacctgaacaaggagtacgaaaacaaatttggcaacattgcggatcttgattattatctgaaagcgattaacttcatcaaaaaagaagtagacgatcccaaattttacgttttctccgacgatattaaatgggctaaagaaaatctgaacctgacggataacgtaacttatgttgaacacaacaaagggagcgactcttacaaagacatgcgtctgatgacctgctgtaaacataacatcatcgccaactctacattctcttggtggggcgcgtttcttaacgagaacaagaacaaaatcgtaatcgcgccgggcaaatggatcaacgttgaaggcgtcggtggcatcaacctgttccctgaaggttggatcgtttactga

SEQ ID NO: 16 - DNA, 900 bp, Artificial Sequence
  Nucleotide sequence encoding Bm2FT_2
atgggttgcataaaaagactattcttatatgaatacggaggacgatgttttttggtaattgttaaaataaaaggtggatttggtaaccaattgtttacatacgctagtgcttatgcaatatctcaagaactgcaacaaaacttaattatggataaggtaatatatgatctagattactttagaaaatttgaattaccttcattatcgttgaagtatgatcaaatgttaattagtaagtttgtacctaatactaaggttaaaactttaatttataaagttttaaggaggttaaaattaaaaggatttacagaggtacatgaaaaaaaggaattttcttttgatgaaaatatttacaatttgtcaggtgatatttatttagatggttattggcagaattatagatatttccataaatattataaagatctgtcggaaatgtttgtaccaagagaaactcctagaaaagaagtaactgattatatcacgtctttacggggagttaattctgttgctatgcatgttaggagaggagattataaaacttttaacggaggaaaatgtttgtctttagattattatattaaggctatggaatatttcaattcaaatgatgtacaattttatgtatttacagatgatattgatttttgtgagaaaaacctcccgaatagtgaaaatattaattatgtgtcaagaagcgagaaacttacagatattgaagaattctttattatgaaagaatgtaaaaattttataattgctaatagtagtttttcgtggtgggctgcttatttaagtgaacagaaagcagatagtttaattgtagcccctgttgttgacatgtggaaaagagatttttatccagatgagtgggtggcattgaatacacatttagaatag

SEQ ID NO: 17 - DNA, 864 bp, Artificial Sequence
  Nucleotide sequence encoding Bm2FT_3
atgataattgttcaaatcaagggcggattaggtaatcaacttttttcgtatgcttctgcttatggaattgcaagagagaatgaaacagaattaattattgatcgatatatatatgatacaagctactctttaagaaaatatatgttggattttttccctgagatcgatgaagcactacttctaaagtatatacctaaaaaaaataaaatttcacaaattatgtataaattgattagaaaatctaagttgaaatataagtacaaagctcaattatttttagaagaagaggaatttaagtttactagaattagtacccagaatgaaaatttgtatttaaatggttattggcaaagttatgtgtactttgataaatatcgtaatgacattattaaaaaattcacccctttagtaagctttaatcaagatggaaatcaacttcttaacgaaattaaaagttataattcagtggctatccatgtcaggagaggggattatattaattttaaaggtggaaagtgtttagatagttcttattatataaaggcaatgaagcatttatacaatttaaaaggaaaaaatttgtttttttatatttttacagatgatgtggaatattgtaaaagaatttttaaaaacgtagctaatgttaaatttataggtgaggaagcaaaattgagtgattttgaagagtttactttgatgactcattgtaaaaacctcataataggtaacagctcattttcttggtgggcagcttacttagcctcttgtaaagataaagctgtaatagctccagtggtagatatgtggactgaagatttctatctacctgaatggataaaaattaaagcggatttacaatag

SEQ ID NO: 18 - DNA, 876 bp, Artificial Sequence
  Nucleotide sequence encoding Bs2FT
atgaaaatagtacacataagtagcggtttaggaaatcaaatgtttcaatatgctctatataaaaaactgtccttaattcaagataatgtttttttggatacaattaccagttatcagttgtatcctaatcaacataatggatatgagttagagaaggtatttacaattaaaccaaggcatgcaagtaaagaattaacatacaatttatcagacttagataattcagtaacatctcgcattcgtaggaaattaattggaagtaaaaagagcatgtatatagaacataaagaatttgaatacgatcctaatttattttatcaagaaaatatatatataaaaggttactggcagaattatgattattttaaagatatagaaaatgaattaaagaatgattttacttttcaaagagctttagatgagaaaaataataatttagctattaaaattaacaatgagaattcaatatcaattcatgtaagacgtggtgattattacttaaacagaaagaatcaagagaagtttggagatatcgctaatttggaatactattcaaaggcaattagctatattaaagaaagaatagacaatccaaagttttatatcttttcagataatgttgagtgggtaaagcaaaatcttaattcgttagaggaagctgtatatatagattataacgtgggaaatgatagttacaaggatatgcaactaatgagtctttgtaaacataatattattgctaatagttcttttagttggtggggagcatttttgaataagaatatggagaaaatagttattgcacctgggaagtggattaatatgaaaggtgtaaaaaaagtcaatcttttcccaaaggattggataatttattaa

SEQ ID NO: 19 - protein, 462 aa, Artificial Sequence
  Amino acid sequence of GTP-mannose-1-phosphate guanylyltransferase
MKLVLLSGGSGKRLWPLSNDTRSKQFLKVLEGRDGQKESMVQRVWSQIEAVGLNESTVIATSKLQRDMITGQVGTDIPLIIEPERRDTFPAIALAASYLHSEEQASEDEIVVVLPVDPYVEDGFFERVKDLESVLRDSKADLALMGVTPTYPSSKYGYIVPEGKVQGDSYFTVDCFTEKPSEEAAVGLINQRALWNCGVFAFRLGYLLQILQEKKLPLQFETLHKEYATLPKISFDYEVVEKASHIVALPYDGYWKDLGTWNTLTEEMATSQIGKGVLTDDSANTHLVNELDIPVTVLGVKDVVVAASPDGILVADKASSPKIKEIIGDWNYPPMYEERLWGWSRVLDYAKYDEETEMVTKRIHISKGKNSTYHYHNLRDEVWTIVRGEGELALDDYIRRVKAGDIIHLPAGKKHGIHALTDLEFIEVQTGKVISNEDSIRLIYDWNDVIKQFQSSRPQVIL

SEQ ID NO: 20 - protein, 359 aa, Artificial Sequence
  Amino acid sequence of phosphomannomurase
LKTIAYYISDYGYGHATRSTAIIRQLLKQNEEIEIIICHSFAIEFLRQSFRYERRVRFREILTDVGYVLKENSLEPDADLLNRQVASYVSSFHTKLMYEKHFMKVANVSFVISDISPLGIAGAYLLKLPSLGISNFTWFTAYEGLIGELSLEFLEKRYKQMTYQFSLACSDEPHWGIKENQSFGFYSREINDSEVQRIRKEIDPEGESYIIYFGLGMKVDIGTLSDLPIWQSPNCKFIVSSNVDVTHPNVYKIPQDETETQHYVAAADLGLTKAGWGTISEAVCAGVPLLITNRSSMKEDRHTIDYLVRHQLCDLIEWKELEGLVVTPSLIETCRRQQINRYKNEAMHIAEEINKKINS

SEQ ID NO: 21 - protein, 313 aa, Artificial Sequence
  Amino acid sequence of GDP-L-fucose synthase
MNKNSKIYVAGHRGLVGSAIVRKLQEKGYSNLVYRTSAELDLRDKPTVDAFFAEEKPEFVFLAAAKVGGIVANNEYPAEFIHDNLLIQSNIIDAAYRNDVEKLLFLGSTCIYPKLAPQPLKEEYLLTGELEPTNEPYAIAKIAGIKMCESYNRQYGTKYISAMPTNLYGPNDNFDLHTSHVLPALLRKFHEAKESNAPFVEMWGTGTPKREFLYSDDLADACVFLMNTYEGNEIVNIGVGEDITIKELGEKVKAVVGYEGNIQFDTSKPDGTPRKLVDVTKLNSLGWKAETALEDGLQKAYQWFLDNELAAAK

SEQ ID NO: 22 - protein, 359 aa, Artificial Sequence
  Amino acid sequence of GDP-D-mannose-4,6-dehydratase
MKTALITGVTGQDGSYLAELLLEKGYEVHGLIRRSSSYNQERLEDLLTEEAASALLNNSNFHLHYGDVTDALNVTRIIGDIQPDEIYNLAAQSHVRVSFDMPGYTLDVDAKGTLNILEAVRILGLTDKTRVYQASTSELYGKVQEVPQKETTPFYPRSPYGVAKIYGFWITKNYRESYSMFAVNGILFNHESERRGETFVTRKITLAASRIAQGKQQKLTLGNLDSLRDWGYAKDYVECMWLILQHDKPEDFVIATGEMHSVREFVQLAFKHTGIEIEWSGEGLEEKGTNKATGEVIVEIDPKFFRPAEVDQLLGDPTKAKTLLKWNPTKTSFEELVRIMVEADMKKVESEEKIKVMFD

SEQ ID NO: 23 - DNA, 1389 bp, Artificial Sequence
  Nucleotide sequence encoding GTP-mannose-1-phosphate guanylyltransferase
atgaaacttgtattgttatcgggtggatctggtaagcgtctatggccgttatcaaatgatacgcgttcgaagcagtttttaaaggtattagaaggacgagatggacagaaagagtcaatggttcagcgcgtctggagtcaaattgaagcggttgggttaaatgagtcaacggttattgcgacgtctaagcttcagcgtgatatgattacaggtcaggttggcaccgatattccgttgattattgaacctgagcgccgcgatacgtttccagcgattgctttagctgcttcatatcttcattccgaagagcaagcatctgaagatgaaatcgttgtggtgttgccagttgacccttatgtggaagacggattttttgaacgggtaaaagatttagaaagtgtgcttcgtgattcaaaagcggatttagcgttaatgggtgttacacctacgtatccttcatctaagtacgggtacatcgtgccggaaggaaaggtacaaggggacagttattttacagtggattgttttacagaaaagccgagtgaagaagcagctgttggattaattaatcagcgtgcgctttggaactgcggcgtttttgcgtttcgtttaggttatttgcttcaaattttacaagagaaaaaacttccacttcaatttgaaacgctacataaagaatatgcaacattgcctaaaattagttttgactatgaagtggtggaaaaggcaagtcatattgtcgcgcttccgtatgatgggtactggaaagatcttggtacatggaatacgttaacggaagaaatggcgacatctcaaattggaaaaggtgtattaacggacgactcagctaatacgcatttagtgaatgaattagatattccggttacggtattaggcgtaaaagatgtagttgttgccgctagtccagatgggatcttagttgcggataaagcatctagtcctaagattaaagaaattattggcgactggaactaccctccaatgtatgaagaacgtctttggggctggtcacgcgtgttagattatgcaaagtatgatgaagaaactgaaatggtgacaaaacgtattcatatttcaaaaggaaagaactcgacgtatcactatcataatttacgtgatgaagtatggacgattgtacgtggagaaggagagcttgcgcttgatgactacattcgccgcgtaaaagcaggggatattattcacttgccggctggcaaaaagcacggaattcatgcgttaaccgaccttgaatttattgaagtacaaacgggaaaagtgatttcaaatgaagatagtattcgccttatttatgactggaatgatgtgatcaagcaattccaatcatcaagaccgcaggtgattttataa

SEQ ID NO: 24 - DNA, 1080 bp, Artificial Sequence
  Nucleotide sequence encoding phosphomannomurase
ttgaaaacaattgcctattacatttcagactacggatatggccacgcgactagaagcacggccattattcgtcaattattaaagcaaaatgaagaaatagaaattattatttgtcattcatttgcgattgagtttctcagacaatcttttagatatgaacgtcgtgtgaggtttcgagagattttaacggatgtcggctacgtgctaaaagaaaattcactagaaccagacgctgatttgttgaatcgtcaagttgcttcttatgtatcaagctttcatacgaagcttatgtatgagaagcactttatgaaagtagccaacgtttcattcgtgatttcggatatttctccgttagggatcgcaggtgcctatctattaaaattgccttctttaggaatatcaaatttcacttggtttacagcatacgaagggttaattggagagctatcgctggaatttttagaaaaacgttataagcagatgacgtatcagttttcgctagcatgtagtgatgagccacattggggtatcaaagaaaatcaaagctttggtttttattcaagagaaataaacgattctgaagtacagcgtattcgtaaagagattgatcctgaaggtgagagttacatcatctacttcggtctgggtatgaaagtagatattggaacgttgtcggacttgcctatttggcaaagtccaaactgcaagtttatcgtttcatcgaatgttgatgttactcatcccaatgtttataaaattcctcaagatgaaacagaaacgcagcactatgtagcagcagctgatcttggtttaacaaaagcaggctggggcacgattagtgaagcggtttgcgctggtgtgccgctgttgattacaaatcgcagcagcatgaaagaagatcgtcatacgattgattatttagttcgtcatcagctatgcgacttaatagagtggaaagagttagaaggtttagtagtaactccttcgcttattgagacatgcaggcggcagcaaatcaatcgctataaaaatgaagcgatgcatatcgccgaagaaatcaataaaaaaataaacagttag

SEQ ID NO: 25 - DNA, 942 bp, Artificial Sequence
  Nucleotide sequence encoding GDP-L-fucose synthase
atgaacaaaaattcgaaaatttacgtagctggtcatagaggtctcgtcggttcagctatcgtacgaaaactacaagaaaaaggctatagcaatctagtgtatcgcacaagcgctgagctagatttaagagacaagccgacagtagacgcattctttgctgaagaaaagccagaatttgttttcttagcagccgctaaagtaggtggtattgtggcaaacaatgaatatccagcggaatttattcacgataacttattgattcaatcaaatattattgatgcagcatatcgcaatgatgtagagaaactattattcctaggaagtacatgtatttatccaaaattagcgcctcagccattaaaagaagaatacttactaacaggtgagctggagccaacaaacgaaccgtatgcaattgctaaaattgctggaatcaaaatgtgtgaatcctataaccgtcagtacggaacaaaatatatctcggcaatgcctactaacctttacggtccaaacgacaattttgaccttcatacatcacacgttcttcctgcactgcttcgtaagttccatgaagcgaaagaaagcaatgcgccgtttgttgaaatgtggggaacaggcacaccaaaacgtgaatttctatattcagatgacctagcagatgcgtgcgtattcttaatgaatacatatgaaggcaatgaaatcgttaatatcggtgtgggagaagatattacgattaaagaacttggcgaaaaagtaaaagcagttgttggttatgaaggaaatattcagtttgatacgtcaaaaccagacggaacgcctcgtaaactagtagacgtaacaaaattgaacagtcttggctggaaagcagaaacagctttagaagacggtcttcaaaaagcgtatcagtggtttttagataacgaactagctgcagcaaaataa

SEQ ID NO: 26 - DNA, 1080 bp, Artificial Sequence
  Nucleotide sequence encoding GDP-D-mannose-4,6-dehydratase
atgaaaacagcattaattacaggtgtaacaggacaagatggatcatacttagcagaacttttactagaaaaaggctatgaagtgcacggactaattcgccgcagctcttcttataaccaagagcgtctagaagatcttttaacagaagaagcagcgagcgcattattaaacaactcaaacttccaccttcactatggtgacgtaacagatgcattaaatgttactcgtattattggtgacattcagccagatgaaatttacaatctagctgcacagtcacatgtacgtgtgtcttttgatatgcctggatatacattagatgttgatgcaaaaggtacgttaaacattcttgaagctgtacgtattttagggttaacagataaaacacgtgtgtaccaagcttctacatctgaactgtacggaaaagttcaagaagtaccacaaaaggaaacaacacctttctaccctcgttctccatatggcgtagcgaaaatttacggcttttggattacaaagaactaccgtgaatcttatagcatgtttgcagtaaacggtattttatttaaccatgaatcagagcgccgcggcgaaacgttcgtaacacgtaaaattacgcttgctgcttcacgtatcgcgcaaggcaagcagcaaaaattaacgcttggaaacttagactctttacgtgactggggttacgcaaaagactatgtagaatgcatgtggttaattcttcaacacgataaacctgaagattttgttattgcgactggtgaaatgcactcagtacgtgaatttgtacagcttgcattcaaacatacaggcattgaaattgagtggagcggtgaaggtctagaagaaaaaggaacaaataaagcaacgggtgaagtgatcgtagaaatcgatcctaagttcttccgtcctgcagaagtggatcaattgttaggtgatccaactaaagccaagactttattaaagtggaaccccactaagacttcgtttgaagaattagttcgcattatggtggaagcggacatgaagaaggttgaaagcgaagagaagattaaggtgatgtttgattaa

SEQ ID NO: 27 - protein, 587 aa, Artificial Sequence
  Amino acid sequence of lactose permease Lac12
MADHSSSSSSLQKKPINTIEHKDTLGNDRDHKEALNSDNDNTSGLKINGVPIEDAREEVLLPGYLSKQYYKLYGLCFITYLCATMQGYDGALMGSIYTEDAYLKYYHLDINSSSGTGLVFSIFNVGQICGAFFVPLMDWKGRKPAILIGCLGVVIGAIISSLTTTKSALIGGRWFVAFFATIANAAAPTYCAEVAPAHLRGKVAGLYNTLWSVGSIVAAFSTYGTNKNFPNSSKAFKIPLYLQMMFPGLVCIFGWLIPESPRWLVGVGREEEAREFIIKYHLNGDRTHPLLDMEMAEIIESFHGTDLSNPLEMLDVRSLFRTRSDRYRAMLVILMAWFGQFSGNNVCSYYLPTMLRNVGMKSVSLNVLMNGVYSIVTWISSICGAFFIDKIGRREGFLGSISGAALALTGLSICTARYEKTKKKSASNGALVFIYLFGGIFSFAFTPMQSMYSTEVSTNLTRSKAQLLNFVVSGVAQFVNQFATPKAMKNIKYWFYVFYVFFDIFEFIVIYFFFVETKGRSLEELEVVFEAPNPRKASVDQAFLAQVRATLVQRNDVRVANAQNLKEQEPLKSDADHVEKLSEAESV

SEQ ID NO: 28 - protein, 413 aa, Artificial Sequence
  Amino acid sequence of lactose permease LacY
MKSSKSLYWKLSAYFFFFFFTWSSSYSLFSIWLGQEIKLNGSATGLIFSVNAIFALCMQPLYGYISDRIGLKKHVLFFISCLLVFVGPFYIFVYGPLLQYNVVIGAIIGGLYLGVAFLAGIGAIETYIEKVSRKYKFEYGKSRMWGSLGWAAATFFAGQLFNINPHINFWVASVSAVILVAIIFSVKVEMSSYEMEKAESVTLRDVGSLFLLKEFWFFMIYVVGVTCVYGVYDQQFPIYYASLFPTESIGNQVFGYLNSFQVFLEAGMMFAAPFIVNKIGAKNSLILAGFLMGFRIIGSGLVVGPIGISSMKLIHALELPIMLIAIFKYLAANFDTRLSSILYLVGFQFASQIGASVLSPIVGGLYDSVGFSRTYLIMGGMVLVFNVISMFTLLNSKKHRFIRKDVQENTQII

SEQ ID NO: 29 - DNA, 1764 bp, Artificial Sequence
  Nucleotide sequence encoding lactose permease Lac12
atggctgatcactcttcttcttcttcttctttacaaaaaaaaccaattaacacaattgaacacaaagatacattaggtaacgatcgtgatcacaaagaagctttaaactctgataacgataacacatctggtttaaaaattaacggtgtaccaattgaagatgctcgtgaagaagtattattaccaggttacttatctaaacaatactacaaattatacggtttatgtttcattacatacttatgtgctacaatgcaaggttacgatggtgctttaatgggttctatttacacagaagatgcttacttaaaatactaccacttagatattaactcttcttctggtacaggtttagtattctctattttcaacgtaggtcaaatttgtggtgctttcttcgtaccattaatggattggaaaggtcgtaaaccagctattttaattggttgtttaggtgtagtaattggtgctattatttcttctttaacaacaacaaaatctgctttaattggtggtcgttggttcgtagctttcttcgctacaattgctaacgctgctgctccaacatactgtgctgaagtagctccagctcacttacgtggtaaagtagctggtttatacaacacattatggtctgtaggttctattgtagctgctttctctacatacggtacaaacaaaaacttcccaaactcttctaaagctttcaaaattccattatacttacaaatgatgttcccaggtttagtatgtattttcggttggttaattccagaatctccacgttggttagtaggtgtaggtcgtgaagaagaagctcgtgaattcattattaaataccacttaaacggtgatcgtacacacccattattagatatggaaatggctgaaattattgaatctttccacggtacagatttatctaacccattagaaatgttagatgtacgttctttattccgtacacgttctgatcgttaccgtgctatgttagtaattttaatggcttggttcggtcaattctctggtaacaacgtatgttcttactacttaccaacaatgttacgtaacgtaggtatgaaatctgtatctttaaacgtattaatgaacggtgtatactctattgtaacatggatttcttctatttgtggtgctttcttcattgataaaattggtcgtcgtgaaggtttcttaggttctatttctggtgctgctttagctttaacaggtttatctatttgtacagctcgttacgaaaaaacaaaaaaaaaatctgcttctaacggtgctttagtattcatttacttattcggtggtattttctctttcgctttcacaccaatgcaatctatgtactctacagaagtatctacaaacttaacacgttctaaagctcaattattaaacttcgtagtatctggtgtagctcaattcgtaaaccaattcgctacaccaaaagctatgaaaaacattaaatactggttctacgtattctacgtattcttcgatattttcgaattcattgtaatttacttcttcttcgtagaaacaaaaggtcgttctttagaagaattagaagtagtattcgaagctccaaacccacgtaaagcttctgtagatcaagctttcttagctcaagtacgtgctacattagtacaacgtaacgatgtacgtgtagctaacgctcaaaacttaaaagaacaagaaccattaaaatctgatgctgatcacgtagaaaaattatctgaagctgaatctgtataa

SEQ ID NO: 30 - DNA, 1242 bp, Artificial Sequence
  Nucleotide sequence encoding lactose permease LacY
atgaaaagttcaaaaagtttatattggaagctgagtgcatattttttcttcttcttttttacgtggtcgtccagctactctttattttctatctggttagggcaagagattaagttgaacggatcagcaacaggcttaatcttttctgtgaacgctatctttgctttgtgtatgcagcctttgtacggatatatatctgacaggataggtttaaagaaacacgttttattttttattagctgtcttttagtgtttgtaggaccattttatatttttgtttatggacctttgcttcaatacaatgtggtgataggggctattattggaggcttatatttaggagtagcgtttttggcgggcatcggagcgattgaaacatacatagagaaagtcagccgaaaatataaatttgagtatggaaaatctagaatgtgggggtcattaggctgggctgcagctacgttttttgcaggacaattatttaatattaatcctcacattaatttttgggtggcatctgtttcagcggttatcctagtcgctattattttttctgtaaaagtagaaatgagcagttatgaaatggaaaaagctgaatccgtcacgctaagagatgtaggtagtttatttttattgaaggaattttggttttttatgatttatgttgttggtgttacatgcgtatatggggtatacgatcagcaatttcctatctattatgcatctttgtttcctactgaatcgataggtaaccaagtatttggctacttaaattcgtttcaagtatttttagaagctggaatgatgttcgcagcaccgtttattgtaaataagatcggtgcaaaaaatagtttaattttagcaggatttctaatgggatttcgtattattgggtcagggcttgttgttggtccaatcggaatatcttcaatgaaactcattcatgcattagaacttcctattatgctcattgccatctttaaatatttggcagctaactttgacacgcgcctatcttccatcctttatttggttggattccaatttgcttcgcaaataggtgcttcagttctttcacccatagtgggaggattatatgatagcgtaggtttttcccgtacctatttaattatgggaggtatggttttggtatttaacgttatttcgatgtttacactactaaactctaaaaaacatagatttataagaaaagatgtacaagaaaacacgcagattatatag

SEQ ID NO: 31 - DNA, 23 bp, Artificial Sequence
  primer Te2FT_F
catatgattatcgttcatctgtg

SEQ ID NO: 32 - DNA, 23 bp, Artificial Sequence
  primer Te2FT_R
ctcgagtcacagaacaatccacc

SEQ ID NO: 33 - DNA, 23 bp, Artificial Sequence
  primer Bt2FT_F
catatgaacgaaatccacgtgct

SEQ ID NO: 34 - DNA, 25 bp, Artificial Sequence
  primer Bt2FT_1_R
ctcgagtcactggccagccggaatc

SEQ ID NO: 35 - DNA, 24 bp, Artificial Sequence
  primer Bm2FT_F
catatgaaaattgttcagatttct

SEQ ID NO: 36 - DNA, 25 bp, Artificial Sequence
  primer Bm2FT_R
ctcgagtcagtaaacgatccaacct

SEQ ID NO: 37 - DNA, 25 bp, Artificial Sequence
  primer Lg2FT_F
catatgctgtacgttgaaatggacg

SEQ ID NO: 38 - DNA, 25 bp, Artificial Sequence
  primer Lg2FT_R
ctcgagttacgcgtcgatcaggatc

SEQ ID NO: 39 - DNA, 24 bp, Artificial Sequence
  primer Ls2FT_F
catatggaagagattcacaccctg

SEQ ID NO: 40 - DNA, 24 bp, Artificial Sequence
  primer Ls2FT_R
ctcgagctaacggccggcaggtac

SEQ ID NO: 41 - DNA, 25 bp, Artificial Sequence
  primer Ll2FT_F
catatgtctaaaaacatttatgtac

SEQ ID NO: 42 - DNA, 26 bp, Artificial Sequence
  primer Ll2FT_R
ctcgagttagattttgatccagttgt

SEQ ID NO: 43 - DNA, 39 bp, Artificial Sequence
  primer Am2FT_1_F
aagaaggagatatacatatgatggctggacattcttgcg

SEQ ID NO: 44 - DNA, 40 bp, Artificial Sequence
  primer Am2FT_1_R
tggtggtggtggtgctcgagttaaatgcgcagccatgagc

SEQ ID NO: 45 - DNA, 39 bp, Artificial Sequence
  primer Am2FT_2_F
aagaaggagatatacatatgatgaacatggaacgtaaga

SEQ ID NO: 46 - DNA, 40 bp, Artificial Sequence
  primer Am2FT_2_R
tggtggtggtggtgctcgagttacagggtcacccagtgcg

SEQ ID NO: 47 - DNA, 38 bp, Artificial Sequence
  primer Fp2FT_F
aagaaggagatatacatatgatgatttacgtggaaatg

SEQ ID NO: 48 - DNA, 39 bp, Artificial Sequence
  primer Fp2FT_R
tggtggtggtggtgctcgagttattcgttaacgatgtta

SEQ ID NO: 49 - DNA, 38 bp, Artificial Sequence
  primer Ri2FT_F
aagaaggagatatacatatgatgatcgcagttaagatc

SEQ ID NO: 50 - DNA, 40 bp, Artificial Sequence
  primer Ri2FT_R
tggtggtggtggtgctcgagttatttcaggataatccagt

SEQ ID NO: 51 - DNA, 39 bp, Artificial Sequence
  primer Bm2FT_2_F
aagaaggagatatacatatgggttgcattaaacgcctgt

SEQ ID NO: 52 - DNA, 40 bp, Artificial Sequence
  primer Bm2FT_2_R
tggtggtggtggtgctcgagctattccaggtgagtgttca

SEQ ID NO: 53 - DNA, 38 bp, Artificial Sequence
  primer Bm2FT_3_F
aagaaggagatatacatatgatcattgtccagattaaa

SEQ ID NO: 54 - DNA, 41 bp, Artificial Sequence
  primer Bm2FT_3_R
tggtggtggtggtgctcgagctattgaagatccgctttgat

SEQ ID NO: 55 - DNA, 38 bp, Artificial Sequence
  primer Bm2FT_4_F
aagaaggagatatacatatgatcattgtgcgtgttatc

SEQ ID NO: 56 - DNA, 40 bp, Artificial Sequence
  primer Bm2FT_4_R
tggtggtggtggtgctcgagttagaacgtattaatacact

SEQ ID NO: 57 - DNA, 38 bp, Artificial Sequence
  primer Bs2FT_F
aagaaggagatatacatatgaaaattgtaaaagttatc

SEQ ID NO: 58 - DNA, 40 bp, Artificial Sequence
  primer Bs2FT_R
tggtggtggtggtgctcgagttagtagatgatccagtctt

SEQ ID NO: 59 - DNA, 36 bp, Artificial Sequence
  primer Gs2FT_F
aagaaggagatatacatatgaaaattgtaaaagtta

SEQ ID NO: 60 - DNA, 39 bp, Artificial Sequence
  primer Gs2FT_R
tggtggtggtggtgctcgagttagattttaatccattct

SEQ ID NO: 61 - DNA, 25 bp, Artificial Sequence
  primer TAG_PET24ma_F
tagctcgagcaccaccaccaccacc

SEQ ID NO: 62 - DNA, 25 bp, Artificial Sequence
  primer TAA_PET24ma_F
taactcgagcaccaccaccaccacc

SEQ ID NO: 63 - DNA, 40 bp, Artificial Sequence
  primer PET24ma_R
catatgtatatctccttcttaaagttaaacaaaattattt